European Patent Application EP 4 722 371 A2, published April 8, 2026. Title: Promoter. Applicant: The University of Bristol. Application EP. The sequence listing filed with the application follows.

SEQUENCE LISTING (63 sequences)

SEQ ID NO: 1 - DNA, 1249 bp, unidentified
  misc_feature 1..1249: note = Exemplary nephrin promoter
  source 1..1249: mol_type = other DNA
cctgcagggcccactagtctgtaatcccagcattttgggaggctgaggcagatggatcacctgaggtcaggagttcgagaccagcctggccaacatgatgaaaccccgtctctagtaaaaatacaaaaattagccaggcatggtgctatatacctgtagtaccagctacttgggagacagaggtgggagaattacttgaacctgggaggttcaagccatgggaggtggaagttgcagtgagccgagatgccactgcactccagcctgagcaacagagcaagactatctcaagaaaaaaaagaaagaaagaaagggacttgccaaggtcatgtatcagggcaaggaagagctgggggcccagctggctgctcccctgctgagctgggagaccaccttgatctgacttctcccatcttcccagcctaagccaggccctggggtcacggaggctggggaggcaccgaggaacgcgcctggcatgtgctgacagggaattttatgctccagctgggccagctgggaggagcctgctgggcagaggccagagctgggggctctggaaggtacctgggggaggttgcactgtgagaatgagctcaagctgggtcagagagcagggctgactctgccagtgcctgcatcagcctcatcgctctcctaggctcctggcctgctggactctgggctgcaggtccttcttgaaaggctgtgagtagtgagacaaggagcaggagtgaggggtggcaggagagaagatagagattgagagagagagagagagagacagagagagaggaagagacagagacaaaaggagagagaacggcttagacaaggagagaaagatggaaagataaagagactgggcgcagtggctcacgcctgtaatcccaacacttggggaggccaaggtgggaggatggcttgaaggaaagagtctgagatcaacctggccaacatagtgagaccccgtctctaaaaaaaaaaaagaaaaaaaaaagaaaaaagaaaaaaaagtttttttaaagagacagagaaagagactcagagattgagactgagagcaagacagagagagacactcacagggaagaggggaagaggaaaacgagaaagggaggagagtaacggaaagagataaaaaagaaaagcaggtggcagagacacagagagagggacccagagaaagccagacagacgcaggtggctggcagcgggcgctgtgggggtcacagtagggggacctgtc

SEQ ID NO: 2 - DNA, 819 bp, unidentified
  misc_feature 1..819: note = Exemplary minimal nephrin promoter
  source 1..819: mol_type = other DNA
ggccctggggtcacggaggctggggaggcaccgaggaacgcgcctggcatgtgctgacagggaattttatgctccagctgggccagctgggaggagcctgctgggcagaggccagagctgggggctctggaaggtacctgggggaggttgcactgtgagaatgagctcaagctgggtcagagagcagggctgactctgccagtgcctgcatcagcctcatcgctctcctaggctcctggcctgctggactctgggctgcaggtccttcttgaaaggctgtgagtagtgagacaaggagcaggagtgaggggtggcaggagagaagatagagattgagagagagagagagagagacagagagagaggaagagacagagacaaaaggagagagaacggcttagacaaggagagaaagatggaaagataaagagactgggcgcagtggctcacgcctgtaatcccaacacttggggaggccaaggtgggaggatggcttgaaggaaagagtctgagatcaacctggccaacatagtgagaccccgtctctaaaaaaaaaaaagaaaaaaaaaagaaaaaagaaaaaaaagtttttttaaagagacagagaaagagactcagagattgagactgagagcaagacagagagagacactcacagggaagaggggaagaggaaaacgagaaagggaggagagtaacggaaagagataaaaaagaaaagcaggtggcagagacacagagagagggacccagagaaagccagacagacgcaggtggctggcagcgggcgctgtgggggtcacagtagggggacctgtc

SEQ ID NO: 3 - DNA, 265 bp, unidentified
  misc_feature 1..265: note = Exemplary minimal nephrin promoter
  source 1..265: mol_type = other DNA
ggccctggggtcacggaggctggggaggcaccgaggaacgcgcctggcatgtgctgacagggaattttatgctccaggagcaagacagagagagacactcacagggaagaggggaagaggaaaacgagaaagggaggagagtaacggaaagagataaaaaagaaaagcaggtggcagagacacagagagagggacccagagaaagccagacagacgcaggtggctggcagcgggcgctgtgggggtcacagtagggggacctgtc

SEQ ID NO: 4 - DNA, 77 bp, unidentified
  misc_feature 1..77: note = Exemplary proximal promoter region
  source 1..77: mol_type = other DNA
ggccctggggtcacggaggctggggaggcaccgaggaacgcgcctggcatgtgctgacagggaattttatgctccag

SEQ ID NO: 5 - DNA, 32 bp, unidentified
  misc_feature 1..32: note = Exemplary core promoter region
  source 1..32: mol_type = other DNA
gagcaagacagagagagacactcacagggaag

SEQ ID NO: 6 - DNA, 156 bp, unidentified
  misc_feature 1..156: note = Exemplary 5'UTR
  source 1..156: mol_type = other DNA
aggggaagaggaaaacgagaaagggaggagagtaacggaaagagataaaaaagaaaagcaggtggcagagacacagagagagggacccagagaaagccagacagacgcaggtggctggcagcgggcgctgtgggggtcacagtagggggacctgtc

SEQ ID NO: 7 - DNA, 188 bp, unidentified
  misc_feature 1..188: note = Exemplary core promoter region and 5'UTR
  source 1..188: mol_type = other DNA
gagcaagacagagagagacactcacagggaagaggggaagaggaaaacgagaaagggaggagagtaacggaaagagataaaaaagaaaagcaggtggcagagacacagagagagggacccagagaaagccagacagacgcaggtggctggcagcgggcgctgtgggggtcacagtagggggacctgtc

SEQ ID NO: 8 - DNA, 554 bp, unidentified
  misc_feature 1..554: note = Exemplary optional promoter region
  source 1..554: mol_type = other DNA
ctgggccagctgggaggagcctgctgggcagaggccagagctgggggctctggaaggtacctgggggaggttgcactgtgagaatgagctcaagctgggtcagagagcagggctgactctgccagtgcctgcatcagcctcatcgctctcctaggctcctggcctgctggactctgggctgcaggtccttcttgaaaggctgtgagtagtgagacaaggagcaggagtgaggggtggcaggagagaagatagagattgagagagagagagagagagacagagagagaggaagagacagagacaaaaggagagagaacggcttagacaaggagagaaagatggaaagataaagagactgggcgcagtggctcacgcctgtaatcccaacacttggggaggccaaggtgggaggatggcttgaaggaaagagtctgagatcaacctggccaacatagtgagaccccgtctctaaaaaaaaaaaagaaaaaaaaaagaaaaaagaaaaaaaagtttttttaaagagacagagaaagagactcagagattgagactga

SEQ ID NO: 9 - DNA, 430 bp, unidentified
  misc_feature 1..430: note = Exemplary optional upstream promoter region
  source 1..430: mol_type = other DNA
cctgcagggcccactagtctgtaatcccagcattttgggaggctgaggcagatggatcacctgaggtcaggagttcgagaccagcctggccaacatgatgaaaccccgtctctagtaaaaatacaaaaattagccaggcatggtgctatatacctgtagtaccagctacttgggagacagaggtgggagaattacttgaacctgggaggttcaagccatgggaggtggaagttgcagtgagccgagatgccactgcactccagcctgagcaacagagcaagactatctcaagaaaaaaaagaaagaaagaaagggacttgccaaggtcatgtatcagggcaaggaagagctgggggcccagctggctgctcccctgctgagctgggagaccaccttgatctgacttctcccatcttcccagcctaagcca

SEQ ID NO: 10 - skipped

SEQ ID NO: 11 - DNA, 17 bp, unidentified
  misc_feature 1..17: note = Exemplary WT1 binding site
  source 1..17: mol_type = other DNA
cggaggctggggaggca

SEQ ID NO: 12 - skipped

SEQ ID NO: 13 - DNA, 30 bp, unidentified
  misc_feature 1..30: note = Exemplary transcription factor binding region
  source 1..30: mol_type = other DNA
gagcaagacagagagagacactcacaggga

SEQ ID NO: 14 - DNA, 1192 bp, unidentified
  misc_feature 1..1192: note = Exemplary variant nephrin promoter
  source 1..1192: mol_type = other DNA
cacctgaggtcaggagttcgagaccagcgtggccaacatgatgaaaccccgtctctagtaaaaatacaaaaattagccaggcatggtgctatatacctgtagcaccagctacttgggagacagaggtgggagaattacttgaacctgggaggttcaagccatgggaggtggaagttgcagtgagccgagatgccactgcactccagcctgagcaacagagcaagactatctcaagaaaagaaagaaagaaagaaagagacttgccaaggtcatgtatcagggcaaggaagagctgggggcccagctggctgctcccctgctgagctgggagaccaccttgatctgacttctcccatcttcccagcctaagccaggccctggggtcacggaggctggggaggcaccgaggaacgcgcctggcatgtgctgacaggggattttatgctccagctgggccagctgggaggagcctgctgggcagaggccagagctgggggctctggaaggtacctgggggaggttgcactgtgagaatgagctcaagctgggtcagagagcagggctgactctgccagtgcctgcatcagcctcatcgctctcctaggctcctggcctgctggactctgggctgcaggtccttcttgaaaggctgtgagtagtgagacaaggagcaggagtgaggggtggcaggagagaagatagagattgagagagagagagagagagagacagagagagaggaagagacagagacaaaaggagagagaacggcttagacaaggagagaaagatggaaagataaagagactgggcgcagtggctcacgcctgtaatcccaacacttggggaggccaaggtgggaggatggcttgaaggaaagagtctgagatcaacctggccaacatagtgagaccccgtctctaaaaaaaaaagaaaaaaaaaagaaaaaagaaaaaaaagtttttttaaagagacagagaaagagactcagagattgagactgagagcaagacagagagagatactcacagggaagaggggaagaggaaaacgagaaagggaggagagtaacggaaagagataaaaaagaaaagcaggtggcagagacacacagagagggacccagagaaagccagacagacgcaggtggctggcagcgggcgctgtgggggtcacagtagggggacctgtg

SEQ ID NO: 15 - DNA, 819 bp, unidentified
  misc_feature 1..819: note = Exemplary minimal nephrin promoter variant
  source 1..819: mol_type = other DNA
ggccctggggtcacggaggctggggaggcaccgaggaacgcgcctggcatgtgctgacaggggattttatgctccagctgggccagctgggaggagcctgctgggcagaggccagagctgggggctctggaaggtacctgggggaggttgcactgtgagaatgagctcaagctgggtcagagagcagggctgactctgccagtgcctgcatcagcctcatcgctctcctaggctcctggcctgctggactctgggctgcaggtccttcttgaaaggctgtgagtagtgagacaaggagcaggagtgaggggtggcaggagagaagatagagattgagagagagagagagagagagacagagagagaggaagagacagagacaaaaggagagagaacggcttagacaaggagagaaagatggaaagataaagagactgggcgcagtggctcacgcctgtaatcccaacacttggggaggccaaggtgggaggatggcttgaaggaaagagtctgagatcaacctggccaacatagtgagaccccgtctctaaaaaaaaaagaaaaaaaaaagaaaaaagaaaaaaaagtttttttaaagagacagagaaagagactcagagattgagactgagagcaagacagagagagatactcacagggaagaggggaagaggaaaacgagaaagggaggagagtaacggaaagagataaaaaagaaaagcaggtggcagagacacacagagagggacccagagaaagccagacagacgcaggtggctggcagcgggcgctgtgggggtcacagtagggggacctgtg

SEQ ID NO: 16 - DNA, 265 bp, unidentified
  misc_feature 1..265: note = Exemplary minimal nephrin promoter variant
  source 1..265: mol_type = other DNA
ggccctggggtcacggaggctggggaggcaccgaggaacgcgcctggcatgtgctgacaggggattttatgctccaggagcaagacagagagagatactcacagggaagaggggaagaggaaaacgagaaagggaggagagtaacggaaagagataaaaaagaaaagcaggtggcagagacacagagagagggacccagagaaagccagacagacgcaggtggctggcagcgggcgctgtgggggtcacagtagggggacctgtc

SEQ ID NO: 17 - DNA, 77 bp, unidentified
  misc_feature 1..77: note = Exemplary variant proximal promoter region
  source 1..77: mol_type = other DNA
ggccctggggtcacggaggctggggaggcaccgaggaacgcgcctggcatgtgctgacaggggattttatgctccag

SEQ ID NO: 18 - DNA, 32 bp, unidentified
  misc_feature 1..32: note = Exemplary variant core promoter region
  source 1..32: mol_type = other DNA
gagcaagacagagagagatactcacagggaag

SEQ ID NO: 19 - DNA, 156 bp, unidentified
  misc_feature 1..156: note = Exemplary variant 5'UTR
  source 1..156: mol_type = other DNA
aggggaagaggaaaacgagaaagggaggagagtaacggaaagagataaaaaagaaaagcaggtggcagagacacacagagagggacccagagaaagccagacagacgcaggtggctggcagcgggcgctgtgggggtcacagtagggggacctgtg

SEQ ID NO: 20 - DNA, 188 bp, unidentified
  misc_feature 1..188: note = Exemplary variant core promoter region and 5'UTR
  source 1..188: mol_type = other DNA
gagcaagacagagagagatactcacagggaagaggggaagaggaaaacgagaaagggaggagagtaacggaaagagataaaaaagaaaagcaggtggcagagacacacagagagggacccagagaaagccagacagacgcaggtggctggcagcgggcgctgtgggggtcacagtagggggacctgtg

SEQ ID NO: 21 - protein, 1670 aa, unidentified
  REGION 1..1670: note = Exemplary COL4A3 amino acid sequence
MSARTAPRPQVLLLPLLLVLLAAAPAASKGCVCKDKGQCFCDGAKGEKGEKGFPGPPGSPGQKGFTGPEGLPGPQGPKGFPGLPGLTGSKGVRGISGLPGFSGSPGLPGTPGNTGPYGLVGVPGCSGSKGEQGFPGLPGTLGYPGIPGAAGLKGQKGAPAKEEDIELDAKGDPGLPGAPGPQGLPGPPGFPGPVGPPGPPGFFGFPGAMGPRGPKGHMGERVIGHKGERGVKGLTGPPGPPGTVIVTLTGPDNRTDLKGEKGDKGAMGEPGPPGPSGLPGESYGSEKGAPGDPGLQGKPGKDGVPGFPGSEGVKGNRGFPGLMGEDGIKGQKGDIGPPGFRGPTEYYDTYQEKGDEGTPGPPGPRGARGPQGPSGPPGVPGSPGSSRPGLRGAPGWPGLKGSKGERGRPGKDAMGTPGSPGCAGSPGLPGSPGPPGPPGDIVFRKGPPGDHGLPGYLGSPGIPGVDGPKGEPGLLCTQCPYIPGPPGLPGLPGLHGVKGIPGRQGAAGLKGSPGSPGNTGLPGFPGFPGAQGDPGLKGEKGETLQPEGQVGVPGDPGLRGQPGRKGLDGIPGTPGVKGLPGPKGELALSGEKGDQGPPGDPGSPGSPGPAGPAGPPGYGPQGEPGLQGTQGVPGAPGPPGEAGPRGELSVSTPVPGPPGPPGPPGHPGPQGPPGIPGSLGKCGDPGLPGPDGEPGIPGIGFPGPPGPKGDQGFPGTKGSLGCPGKMGEPGLPGKPGLPGAKGEPAVAMPGGPGTPGFPGERGNSGEHGEIGLPGLPGLPGTPGNEGLDGPRGDPGQPGPPGEQGPPGRCIEGPRGAQGLPGLNGLKGQQGRRGKTGPKGDPGIPGLDRSGFPGETGSPGIPGHQGEMGPLGQRGYPGNPGILGPPGEDGVIGMMGFPGAIGPPGPPGNPGTPGQRGSPGIPGVKGQRGTPGAKGEQGDKGNPGPSEISHVIGDKGEPGLKGFAGNPGEKGNRGVPGMPGLKGLKGLPGPAGPPGPRGDLGSTGNPGEPGLRGIPGSMGNMGMPGSKGKRGTLGFPGRAGRPGLPGIHGLQGDKGEPGYSEGTRPGPPGPTGDPGLPGDMGKKGEMGQPGPPGHLGPAGPEGAPGSPGSPGLPGKPGPHGDLGFKGIKGLLGPPGIRGPPGLPGFPGSPGPMGIRGDQGRDGIPGPAGEKGETGLLRAPPGPRGNPGAQGAKGDRGAPGFPGLPGRKGAMGDAGPRGPTGIEGFPGPPGLPGAIIPGQTGNRGPPGSRGSPGAPGPPGPPGSHVIGIKGDKGSMGHPGPKGPPGTAGDMGPPGRLGAPGTPGLPGPRGDPGFQGFPGVKGEKGNPGFLGSIGPPGPIGPKGPPGVRGDPGTLKIISLPGSPGPPGTPGEPGMQGEPGPPGPPGNLGPCGPRGKPGKDGKPGTPGPAGEKGNKGSKGEPGPAGSDGLPGLKGKRGDSGSPATWTTRGFVFTRHSQTTAIPSCPEGTVPLYSGFSFLFVQGNQRAHGQDLGTLGSCLQRFTTMPFLFCNVNDVCNFASRNDYSYWLSTPALMPMNMAPITGRALEPYISRCTVCEGPAIAIAVHSQTTDIPPCPHGWISLWKGFSFIMFTSAGSEGTGQALASPGSCLEEFRASPFLECHGRGTCNYYSNSYSFWLASLNPERMFRKPIPSTVKAGELEKIISRCQVCMKKRH

SEQ ID NO: 22 - protein, 1690 aa, unidentified
  REGION 1..1690: note = Exemplary COL4A4 amino acid sequence
MWSLHIVLMRCSFRLTKSLATGPWSLILILFSVQYVYGSGKKYIGPCGGRDCSVCHCVPEKGSRGPPGPPGPQGPIGPLGAPGPIGLSGEKGMRGDRGPPGAAGDKGDKGPTGVPGFPGLDGIPGHPGPPGPRGKPGMSGHNGSRGDPGFPGGRGALGPGGPLGHPGEKGEKGNSVFILGAVKGIQGDRGDPGLPGLPGSWGAGGPAGPTGYPGEPGLVGPPGQPGRPGLKGNPGVGVKGQMGDPGEVGQQGSPGPTLLVEPPDFCLYKGEKGIKGIPGMVGLPGPPGRKGESGIGAKGEKGIPGFPGPRGDPGSYGSPGFPGLKGELGLVGDPGLFGLIGPKGDPGNRGHPGPPGVLVTPPLPLKGPPGDPGFPGRYGETGDVGPPGPPGLLGRPGEACAGMIGPPGPQGFPGLPGLPGEAGIPGRPDSAPGKPGKPGSPGLPGAPGLQGLPGSSVIYCSVGNPGPQGIKGKVGPPGGRGPKGEKGNEGLCACEPGPMGPPGPPGLPGRQGSKGDLGLPGWLGTKGDPGPPGAEGPPGLPGKHGASGPPGNKGAKGDMVVSRVKGHKGERGPDGPPGFPGQPGSHGRDGHAGEKGDPGPPGDHEDATPGGKGFPGPLGPPGKAGPVGPPGLGFPGPPGERGHPGVPGHPGVRGPDGLKGQKGDTISCNVTYPGRHGPPGFDGPPGPKGFPGPQGAPGLSGSDGHKGRPGTPGTAEIPGPPGFRGDMGDPGFGGEKGSSPVGPPGPPGSPGVNGQKGIPGDPAFGHLGPPGKRGLSGVPGIKGPRGDPGCPGAEGPAGIPGFLGLKGPKGREGHAGFPGVPGPPGHSCERGAPGIPGQPGLPGYPGSPGAPGGKGQPGDVGPPGPAGMKGLPGLPGRPGAHGPPGLPGIPGPFGDDGLPGPPGPKGPRGLPGFPGFPGERGKPGAEGCPGAKGEPGEKGMSGLPGDRGLRGAKGAIGPPGDEGEMAIISQKGTPGEPGPPGDDGFPGERGDKGTPGMQGRRGEPGRYGPPGFHRGEPGEKGQPGPPGPPGPPGSTGLRGFIGFPGLPGDQGEPGSPGPPGFSGIDGARGPKGNKGDPASHFGPPGPKGEPGSPGCPGHFGASGEQGLPGIQGPRGSPGRPGPPGSSGPPGCPGDHGMPGLRGQPGEMGDPGPRGLQGDPGIPGPPGIKGPSGSPGLNGLHGLKGQKGTKGASGLHDVGPPGPVGIPGLKGERGDPGSPGISPPGPRGKKGPPGPPGSSGPPGPAGATGRAPKDIPDPGPPGDQGPPGPDGPRGAPGPPGLPGSVDLLRGEPGDCGLPGPPGPPGPPGPPGYKGFPGCDGKDGQKGPVGFPGPQGPHGFPGPPGEKGLPGPPGRKGPTGLPGPRGEPGPPADVDDCPRIPGLPGAPGMRGPEGAMGLPGMRGPSGPGCKGEPGLDGRRGVDGVPGSPGPPGRKGDTGEDGYPGGPGPPGPIGDPGPKGFGPGYLGGFLLVLHSQTDQEPTCPLGMPRLWTGYSLLYLEGQEKAHNQDLGLAGSCLPVFSTLPFAYCNIHQVCHYAQRNDRSYWLASAAPLPMMPLSEEAIRPYVSRCAVCEAPAQAVAVHSQDQSIPPCPQTWRSLWIGYSFLMHTGAGDQGGGQALMSPGSCLEDFRAAPFLECQGRQGTCHFFANKYSFWLTTVKADLQFSSAPAPDTLKESQAQRQKISRCQVCVKYS

SEQ ID NO: 23 - protein, 1685 aa, unidentified
  REGION 1..1685: note = Exemplary COL4A5 amino acid sequence
MKLRGVSLAAGLFLLALSLWGQPAEAAACYGCSPGSKCDCSGIKGEKGERGFPGLEGHPGLPGFPGPEGPPGPRGQKGDDGIPGPPGPKGIRGPPGLPGFPGTPGLPGMPGHDGAPGPQGIPGCNGTKGERGFPGSPGFPGLQGPPGPPGIPGMKGEPGSIIMSSLPGPKGNPGYPGPPGIQGLPGPTGIPGPIGPPGPPGLMGPPGPPGLPGPKGNMGLNFQGPKGEKGEQGLQGPPGPPGQISEQKRPIDVEFQKGDQGLPGDRGPPGPPGIRGPPGPPGGEKGEKGEQGEPGKRGKPGKDGENGQPGIPGLPGDPGYPGEPGRDGEKGQKGDTGPPGPPGLVIPRPGTGITIGEKGNIGLPGLPGEKGERGFPGIQGPPGLPGPPGAAVMGPPGPPGFPGERGQKGDEGPPGISIPGPPGLDGQPGAPGLPGPPGPAGPHIPPSDEICEPGPPGPPGSPGDKGLQGEQGVKGDKGDTCFNCIGTGISGPPGQPGLPGLPGPPGSLGFPGQKGEKGQAGATGPKGLPGIPGAPGAPGFPGSKGEPGDILTFPGMKGDKGELGSPGAPGLPGLPGTPGQDGLPGLPGPKGEPGGITFKGERGPPGNPGLPGLPGNIGPMGPPGFGPPGPVGEKGIQGVAGNPGQPGIPGPKGDPGQTITQPGKPGLPGNPGRDGDVGLPGDPGLPGQPGLPGIPGSKGEPGIPGIGLPGPPGPKGFPGIPGPPGAPGTPGRIGLEGPPGPPGFPGPKGEPGFALPGPPGPPGLPGFKGALGPKGDRGFPGPPGPPGRTGLDGLPGPKGDVGPNGQPGPMGPPGLPGIGVQGPPGPPGIPGPIGQPGLHGIPGEKGDPGPPGLDVPGPPGERGSPGIPGAPGPIGPPGSPGLPGKAGASGFPGTKGEMGMMGPPGPPGPLGIPGRSGVPGLKGDDGLQGQPGLPGPTGEKGSKGEPGLPGPPGPMDPNLLGSKGEKGEPGLPGIPGVSGPKGYQGLPGDPGQPGLSGQPGLPGPPGPKGNPGLPGQPGLIGPPGLKGTIGDMGFPGPQGVEGPPGPSGVPGQPGSPGLPGQKGDKGDPGISSIGLPGLPGPKGEPGLPGYPGNPGIKGSVGDPGLPGLPGTPGAKGQPGLPGFPGTPGPPGPKGISGPPGNPGLPGEPGPVGGGGHPGQPGPPGEKGKPGQDGIPGPAGQKGEPGQPGFGNPGPPGLPGLSGQKGDGGLPGIPGNPGLPGPKGEPGFHGFPGVQGPPGPPGSPGPALEGPKGNPGPQGPPGRPGLPGPEGPPGLPGNGGIKGEKGNPGQPGLPGLPGLKGDQGPPGLQGNPGRPGLNGMKGDPGLPGVPGFPGMKGPSGVPGSAGPEGEPGLIGPPGPPGLPGPSGQSIIIKGDAGPPGIPGQPGLKGLPGPQGPQGLPGPTGPPGDPGRNGLPGFDGAGGRKGDPGLPGQPGTRGLDGPPGPDGLQGPPGPPGTSSVAHGFLITRHSQTTDAPQCPQGTLQVYEGFSLLYVQGNKRAHGQDLGTAGSCLRRFSTMPFMFCNINNVCNFASRNDYSYWLSTPEPMPMSMQPLKGQSIQPFISRCAVCEAPAVVIAVHSQTIQIPHCPQGWDSLWIGYSFMMHTSAGAEGSGQALASPGSCLEEFRSAPFIECHGRGTCNYYANSYSFWLATVDVSDMFSKPQSETLKAGDLRTRISRCQVCMKRT

SEQ ID NO: 24 - DNA, 5013 bp, unidentified
  misc_feature 1..5013: note = Exemplary COL4A3 transgene sequence
  source 1..5013: mol_type = other DNA
atgagcgcccggaccgcccccaggccgcaggtgctcctgctgccgctcctgctggtgctcctggcggcggcgcccgcagccagcaagggttgtgtctgtaaagacaaaggccagtgcttctgtgacggggccaaaggggagaagggggagaagggctttcctggaccccccggttctcctggccagaaaggattcacaggtcctgaaggcttgcctggaccgcagggacccaagggctttccaggacttccaggactcacgggttccaaaggtgtaaggggaataagtggattgccaggattttctggttctcctggacttccaggcaccccaggcaataccgggccttacggacttgtcggtgtaccaggatgcagtggttctaagggtgagcaggggtttccaggactcccagggacactgggctacccagggatcccgggtgctgctggtttgaaaggacaaaagggtgctcctgctaaagaagaagatatagaacttgatgcaaaaggcgaccccgggttgccaggggctccaggaccccagggtttgccaggccctccaggttttcctgggcctgttggcccacctggtcctccgggattctttggctttccaggagccatgggacctagaggacctaagggtcacatgggtgaaagagtgataggacataaaggagagcggggtgtgaaagggttaacaggacccccgggaccaccaggaacagttattgtgaccctaactggcccagataacagaacggacctcaagggggaaaagggagacaagggagcaatgggcgagcctggacctcctggaccctcaggactgcctggagaatcatatggatctgaaaagggtgctcctggagaccctggcctgcagggaaaacccggaaaagatggtgttcctggcttccctggaagtgagggagtcaagggcaacaggggtttccctgggttaatgggtgaagatggcattaagggacagaaaggggacattggccctccaggatttcgtggtccaacagaatattatgacacataccaggaaaagggagatgaaggcactccaggcccaccagggcccagaggagctcgtggcccacaaggtcccagtggtccccccggagttcctggaagtcctggatcatcaaggcctggcctcagaggagcccctggatggccaggcctgaaaggaagtaaaggggaacgaggccgcccaggaaaggatgccatggggactcctgggtccccaggttgtgctggttcaccaggtcttccaggatcaccgggacctccaggaccgccaggtgacatcgtttttcgcaagggtccacctggagatcacggactgccaggctatctagggtctccaggaatcccaggagttgatgggcccaaaggagaaccaggcctcctgtgtacacagtgcccttatatcccagggcctcccggtctcccaggattgccagggttacatggtgtaaaaggaatcccaggaagacaaggcgcagctggcttgaaaggaagcccagggtccccaggaaatacaggtcttccaggatttccaggtttcccaggtgcccagggtgacccaggacttaaaggagaaaaaggtgaaacacttcagcctgaggggcaagtgggtgtcccaggtgacccggggctcagaggccaacctgggagaaagggcttggatggaattcctggaactccgggagtgaaaggattaccaggacctaaaggcgaactggctctgagtggtgagaaaggggaccaaggtcctccaggggatcctggctcccctgggtccccaggacctgcaggaccagctggaccacctggctacggaccccaaggagaacctggtctccagggcacgcaaggagttcctggagcccccggaccacccggagaagccggccctaggggagagctcagtgtttcaacaccagttccaggcccaccaggacctccagggccccctggccatcctggcccccaaggtccacctggtatccctggatccctggggaaatgtggagatcctggtcttccagggcctgatggtgaaccaggaattccaggaattggatttcctgggcctcctggacctaagggagaccaaggttttccaggtacaaaaggatcactgggttgtcctggaaaaatgggagagcctgggttacctggaaagccaggcctcccaggagccaagggagaaccagcagtagccatgcctggaggaccaggaacaccaggttttccaggagaaagaggcaattctggggaacatggagaaattggactccctggacttccaggtctccctggaactccaggaaatgaagggcttgatggaccacgaggagatccagggcagcctggaccacctggagaacaaggacccccaggaaggtgcatagagggtcccaggggagcccaaggacttccaggcttaaatggattgaaagggcaacaaggcagaagaggtaaaacggggccaaagggagacccaggaattccaggcttggatagatcaggatttcctggagaaactggatcaccaggaattccaggtcatcaaggtgaaatgggaccactgggtcaaagaggatatccaggaaatccgggaattttagggccaccaggtgaagatggagtgattgggatgatgggctttcctggagccattggccctccagggccccctgggaacccaggcacaccagggcagagggggagccctggaattccaggagtaaagggccagagaggaaccccaggagccaagggggaacaaggagataaaggaaatcccgggccttcagagatatcccacgtaataggggacaaaggagaaccaggtctcaaaggattcgcaggaaatccaggtgagaaaggaaacagaggcgttccagggatgccaggtttaaagggcctcaaaggactacccggaccagcaggaccaccaggccccagaggagatttgggcagcactgggaatcctggagaaccaggactgcgtggtataccaggaagcatggggaacatgggcatgccaggttctaaaggaaaaaggggaactttgggattcccaggtcgagcaggaagaccaggcctcccaggtattcatggtctccagggagataagggagagccaggttattcagaaggtacaaggccaggaccaccgggaccaacgggggatccaggactgccgggtgatatgggaaagaaaggagaaatggggcaacctggcccacctggacatttggggcctgctggacctgagggagcccctggaagtcctggaagtcctggcctcccaggaaagccaggtcctcatggtgatttgggttttaaaggaatcaaaggcctcctgggccctccaggaatcagaggccctccaggtcttccaggatttccaggatctcctggaccaatgggtataagaggtgaccaaggacgtgatggaattcctggtccagccggagaaaagggagaaacgggtttattgagggcccctccaggcccaagagggaaccctggtgctcaaggagccaaaggagacaggggagccccaggttttcctggcctcccgggcagaaaaggggccatgggagatgctggacctcgaggacccacaggcatagaaggattcccagggccaccaggtctgcccggtgcaattatccctggccagacaggaaatcgtggtccaccaggctcaagaggaagcccaggtgcgcctggtccccctggacctccagggagtcatgtaataggcataaaaggagacaaagggtctatgggccaccctggcccaaaaggtccacctggaactgcaggagacatgggaccaccaggtcgtctgggagcaccaggtactccaggtcttccaggacccagaggtgatcctggattccaggggtttccaggcgtgaaaggagaaaagggtaatcctggatttctaggatccattggacctccaggaccaattgggccaaaaggaccacctggtgtacgtggagaccctggcacacttaagattatctcccttccaggaagcccagggccacctggcacacctggagaaccagggatgcagggagaacctgggccaccagggccacctggaaacctaggaccctgtgggccaagaggtaagccaggcaaggatggaaaaccaggaactcctggaccagctggagaaaaaggcaacaaaggttctaaaggagagccaggaccagctggatcagatggattgccaggtttgaaaggaaaacgtggagacagtggatcacctgcaacctggacaacgagaggctttgtcttcacccgacacagtcaaaccacagcaattccttcatgtccagaggggacagtgccactctacagtgggttttcttttctttttgtacaaggaaatcaacgagcccacggacaagaccttggaactcttggcagctgcctgcagcgatttaccacaatgccattcttattctgcaatgtcaatgatgtatgtaattttgcatctcgaaatgattattcatactggctgtcaacaccagctctgatgccaatgaacatggctcccattactggcagagcccttgagccttatataagcagatgcactgtttgtgaaggtcctgcgatcgccatagccgttcacagccaaaccactgacattcctccatgtcctcacggctggatttctctctggaaaggattttcattcatcatgttcacaagtgcaggttctgagggcaccgggcaagcactggcctcccctggctcctgcctggaagaattccgagccagcccatttctagaatgtcatggaagaggaacgtgcaactactattcaaattcctacagtttctggctggcttcattaaacccagaaagaatgttcagaaagcctattccatcaactgtgaaagctggggaattagaaaaaataataagtcgctgtcaggtgtgcatgaagaaaagacactga

SEQ ID NO: 25 - DNA, 5073 bp, unidentified
  misc_feature 1..5073: note = Exemplary COL4A4 transgene sequence
  source 1..5073: mol_type = other DNA
atgtggtctctgcacatagtactaatgaggtgctccttcagattgaccaagtccttggccacaggtccctggtcacttatactcattctcttttctgtacaatatgtatatgggagtggaaagaaatacattggtccttgtggaggaagagattgctctgtttgccactgtgttcctgaaaaggggtctcggggtccaccaggaccaccagggccacagggtccaattggacccctgggagccccaggacccattgggctttcaggagagaaaggaatgagaggggaccgcggccctcctggagcagcaggggacaaaggagataagggtccaactggtgttcctggatttccaggtttagatggcatacctgggcacccagggcctcctggacccagaggcaaacctggtatgagtggccacaatggctcaagaggtgacccagggtttccaggaggaagaggagctcttggcccaggaggccccctaggccatcctggggaaaagggagaaaaaggaaattcagtgttcattttaggtgccgttaaaggtattcagggagacagaggggacccaggactgcctggcttaccaggatcttggggtgcaggaggaccggcaggtcccacaggatatcctggagagccagggttagtgggacctccgggccaaccagggcgtccaggtttgaagggaaatcccggtgtgggagtaaaggggcaaatgggagacccgggtgaggttggtcagcaaggttctcctggacccaccctgttggtagagccacctgacttttgtctctataaaggagaaaagggtataaaaggaattcctggaatggttggactgccaggaccaccaggacgcaagggagaatctggtattggggcaaaaggagaaaaaggtattcctggatttccagggcctcggggggatcctggttcctatggatctccaggttttccaggattaaagggagaactaggactggttggagatcctgggctatttggattaattggcccaaagggggatcctggaaatcgagggcacccaggaccaccaggtgttttggtgactccacctcttccactcaaaggcccaccaggggacccagggttccctggccgctatggagaaacaggggatgttggaccacctggtcccccaggtctcttgggcagaccaggggaagcctgtgcaggcatgataggaccccctgggccacaaggatttcctggtcttcctgggcttccaggagaagctggtattcctgggagacctgattctgctccaggaaaaccagggaagccaggatcacctggcttgcctggagcaccaggcctgcagggcctcccaggatcaagtgtgatatactgtagtgttgggaaccccggaccacaaggaataaaaggcaaagttggtcccccaggaggaagaggcccaaaaggagaaaaaggaaatgaaggactctgtgcctgtgagcctggacccatgggcccccctggccctccaggacttcctgggaggcaggggagtaagggagacttggggctccctggctggcttggaacaaaaggtgacccaggacctcctggtgctgaaggacctccagggctaccaggaaagcatggtgcctctggaccacctggcaacaaaggggcgaagggtgacatggttgtatcaagagttaaagggcacaaaggagaaagaggtcctgatgggcccccaggatttccagggcagccaggatcacatggtcgggatggacatgctggagaaaaaggggatccaggacctccaggggatcatgaagatgcgaccccaggtggtaaaggatttcctggacctctgggccccccaggcaaagcaggacctgtggggcccccaggactgggatttcctggtccaccaggagagcgaggccacccaggagttccaggccacccaggtgtgaggggccctgatggcttgaagggtcagaaaggtgacacaatttcttgcaacgtaacctaccctgggaggcatggccctccaggttttgatggacctccaggtccgaagggatttccaggtccccaaggtgcccctgggctgagtggttcagatgggcataaaggcagacctggcacaccaggaacagcggaaataccaggtccacctggttttcgtggtgacatgggagatccgggttttggaggtgaaaaggggtcctcccctgttgggcccccaggccctcccggctcaccaggagtgaatggtcagaaaggaatcccgggagaccctgcatttggtcacctgggacccccgggaaagaggggtctttcaggagtgccagggataaaaggacccagaggtgatccgggatgtccaggggctgaagggccagctggcattcctggattcctaggtctcaaaggtcccaaaggcagagagggacatgctgggtttccaggtgtcccaggtccacctggccattcctgtgaaagaggtgctccagggataccagggcaaccgggactccctgggtatccaggtagcccaggtgctccaggtgggaaaggacagccgggagatgtggggcctcccgggccagctggaatgaaaggcctccccggactcccaggacggcctggggcacatggtcccccaggcctcccaggaatcccaggtccctttggagatgatgggctacctggtcctccaggtccaaagggaccccgggggctgcctggtttcccaggttttcccggagaaagaggaaagcctggtgcagagggatgtcctggcgcaaagggagaacctggagagaagggcatgtctggccttcctggagaccggggactgagaggggccaaaggagccataggacctcccggagatgaaggagaaatggctatcatttcacaaaagggaacacctggggaacctggacctcctggagatgatggattcccaggagaaagaggtgataaaggaactcccgggatgcaagggagaagaggagagccgggaagatacggaccacctggatttcacagaggggaacctggtgagaaaggtcagccagggcctcctggacccccaggccctccaggctcaactggtctaagagggttcattggttttccaggacttccaggtgaccagggtgagccaggttctccaggtccccctggattttcaggaattgatggagcaagaggacctaaaggaaacaaaggtgaccctgccagtcactttggtccacctggtccaaagggtgagccaggtagccctggatgtccagggcattttggagcatccggagagcagggcttgcctggtattcaagggcccagaggatcacctggaaggccagggccacctggctcctctggaccaccagggtgcccaggtgatcacgggatgcctgggctgaggggacagccaggagaaatgggagaccctgggccaagaggcctccagggggatccagggataccaggtcctccgggaataaaaggtccctccggatcacctggcctgaacggcttgcatggattgaaaggtcagaaaggaactaaaggtgcttcaggtttgcatgatgtggggccacctggtccagtgggaatacctgggctaaaaggggagagaggagaccctgggagcccaggaatctctcctccaggtcctcgtggaaagaaaggtcccccaggacccccagggagttcaggaccacctggtcctgcaggtgccacaggaagagctcctaaggacattcctgacccgggtccacctggagatcagggacctcctggtcctgatggcccaagaggagcacctgggcctccaggcctccctgggagtgttgaccttctgagaggggagccaggtgactgtggtctaccagggccaccaggtccccctggcccaccaggccctccaggatacaaaggctttccaggatgtgatggaaaagatggccagaaaggaccagtgggattcccgggaccgcagggaccacatggatttcctgggccacctggagagaagggtttacctggacctccagggagaaaagggcccactggtcttccgggtcccagaggtgaaccggggccacctgcagatgtggatgactgtccccgaatcccaggccttcctggggcgccaggcatgagaggaccagaaggagccatggggctccctggaatgagaggcccctcaggaccagggtgcaaaggagagcctgggctggatggcaggaggggtgtggatggcgtccctgggtctcctgggcctcccggacgtaaaggtgacacaggagaagacggctaccctggaggaccagggcctcctggtcccattggggatcctgggcccaaagggtttggccctggatacctcggtggcttcctcctggttctccacagtcagacggaccaggagcccacctgccccctgggcatgcccaggctctggactgggtatagtctgttatacctggaagggcaagagaaagctcacaatcaagaccttggtctggcagggtcttgccttcccgtatttagcacgctgccctttgcctactgcaacatccaccaggtgtgccactatgcccagagaaacgacagatcctactggctggccagcgctgcgcccctccccatgatgccactctctgaagaggcgatccgcccctatgtcagccgctgtgcggtatgcgaggccccggcccaggcggtggcggtgcacagccaggaccagtccatccccccatgtccgcagacctggaggagcctctggatcgggtattcattcctgatgcacacaggagctggggaccaaggaggagggcaggcccttatgtcacctggcagctgcctggaagatttcagagcagcaccattccttgaatgccagggccggcagggaacttgccactttttcgcaaataagtatagcttctggctcacaacggtgaaagcagacttgcagttttcctctgctccagcaccagacaccttaaaagaaagccaggcccaacgccagaaaatcagccggtgccaggtctgcgtgaagtatagctag

SEQ ID NO: 26 - DNA, 5058 bp, unidentified
  misc_feature 1..5058: note = Exemplary COL4A5 transgene sequence
  source 1..5058: mol_type = other DNA
atgaaactgcgtggagtcagcctggctgccggcttgttcttactggccctgagtctttgggggcagcctgcagaggctgcggcttgctatgggtgttctccaggatcaaagtgtgactgcagtggcataaaaggggaaaagggagagagagggtttccaggtttggaaggacacccaggattgcctggatttccaggtccagaagggcctccggggcctcggggacaaaagggtgatgatggaattccagggccaccaggaccaaaaggaatcagaggtcctcctggacttcctggatttccagggacaccaggtcttcctggaatgccaggccacgatggggccccaggacctcaaggtattcccggatgcaatggaaccaagggagaacgtggatttccaggcagtcccggttttcctggtttacagggtcctccaggaccccctgggatcccaggtatgaagggtgaaccaggtagtataattatgtcatcactgccaggaccaaagggtaatccaggatatccaggtcctcctggaatacaaggcctacctggtcccactggtataccagggccaattggtcccccaggaccaccaggtttgatgggccctcctggtccaccaggacttccaggacctaaggggaatatgggcttaaatttccagggacccaaaggtgaaaaaggtgagcaaggtcttcagggcccacctgggccacctgggcagatcagtgaacagaaaagaccaattgatgtagagtttcagaaaggagatcagggacttcctggtgaccgagggcctcctggacctccagggatacgtggtcctccaggtcccccaggtggtgagaaaggtgagaagggtgagcaaggagagccaggcaaaagaggtaaaccaggcaaagatggagaaaatggccaaccaggaattcctggtttgcctggtgatcctggttaccctggtgaacccggaagggatggtgaaaagggccaaaaaggtgacactggcccacctggacctcctggacttgtaattcctagacctgggactggtataactataggagaaaaaggaaacattgggttgcctgggttgcctggagaaaaaggagagcgaggatttcctggaatacagggtccacctggccttcctggacctccaggggctgcagttatgggtcctcctggccctcctggatttcctggagaaaggggtcagaaaggtgatgaaggaccacctggaatttccattcctggacctcctggacttgacggacagcctggggctcctgggcttccagggcctcctggccctgctggccctcacattcctcctagtgatgagatatgtgaaccaggccctccaggccccccaggatctccaggtgataaaggactccaaggagaacaaggagtgaaaggtgacaaaggtgacacttgcttcaactgcattggaactggtatttcagggcctccaggtcaacctggtttgccaggtctcccaggtcctccaggatctcttggtttccctggacagaaaggggaaaaaggacaagctggtgcaactggtcccaaaggattaccaggcattccaggagctccaggtgctccaggctttcctggatctaaaggtgaacctggtgatatcctcacttttccaggaatgaagggtgacaaaggagagttgggttcccctggagctccagggcttcctggtttacctggcactcctggacaggatggattgccagggcttcctggcccgaaaggagagcctggtggaattacttttaagggtgaaagaggtccccctgggaacccaggtttaccaggcctcccagggaatatagggcctatgggtccccctggtttcggccctccaggcccagtaggtgaaaaaggcatacaaggtgtggcaggaaatccaggccagccaggaataccaggtcctaaaggggatccaggtcagactataacccagccggggaagcctggcttgcctggtaacccaggcagagatggtgatgtaggtcttccaggtgaccctggacttccagggcaaccaggcttgccagggatacctggtagcaaaggagaaccaggtatccctggaattgggcttcctggaccacctggtcccaaaggctttcctggaattccaggacctccaggagcacctgggacacctggaagaattggtctagaaggccctcctgggccacccggctttccaggaccaaagggtgaaccaggatttgcattacctgggccacctgggccaccaggacttccaggtttcaaaggagcacttggtccaaaaggtgatcgtggtttcccaggacctccgggtcctccaggacgcactggcttagatgggctccctggaccaaaaggtgatgttggaccaaatggacaacctggaccaatgggacctcctgggctgccaggaataggtgttcagggaccaccaggaccaccagggattcctgggccaataggtcaacctggtttacatggaataccaggagagaagggggatccaggacctcctggacttgatgttccaggacccccaggtgaaagaggcagtccagggatccccggagcacctggtcctataggacctccaggatcaccagggcttccaggaaaagcaggtgcctctggatttccaggtaccaaaggtgaaatgggtatgatgggacctccaggcccaccaggacctttgggaattcctggcaggagtggtgtacctggtcttaaaggtgatgatggcttgcagggtcagccaggacttcctggccctacaggagaaaaaggtagtaaaggagagcctggccttccaggccctcctggaccaatggatccaaatcttctgggctcaaaaggagagaagggggaacctggcttaccaggtatacctggagtttcagggccaaaaggttatcagggtttgcctggagacccagggcaacctggactgagtggacaacctggattaccaggaccaccaggtcccaaaggtaaccctggtctccctggacagccaggtcttataggacctcctggacttaaaggaaccatcggtgatatgggttttccagggcctcagggtgtggaagggcctcctggaccttctggagttcctggacaacctggctccccaggattacctggacagaaaggcgacaaaggtgatcctggtatttcaagcattggtcttccaggtcttcctggtccaaagggtgagcctggtctgcctggatacccagggaaccctggtatcaaaggttctgtgggagatcctggtttgcccggattaccaggaacccctggagcaaaaggacaaccaggccttcctggattcccaggaaccccaggccctcctggaccaaaaggtattagtggccctcctgggaaccccggccttccaggagaacctggtcctgtaggtggtggaggtcatcctgggcaaccagggcctccaggcgaaaaaggcaaacccggtcaagatggtattcctggaccagctggacagaagggtgaaccaggtcaaccaggctttggaaacccaggaccccctggacttccaggactttctggccaaaagggtgatggaggattacctgggattccaggaaatcctggccttccaggtccaaagggcgaaccaggctttcacggtttccctggtgtgcagggtcccccaggccctcctggttctccgggtccagctctggaaggacctaaaggcaaccctgggccccaaggtcctcctgggagaccaggtctaccaggtccagaaggtcctccaggtctccctggaaatggaggtattaaaggagagaagggaaatccaggccaacctgggctacctggcttgcctggtttgaaaggagatcaaggaccaccaggactccagggtaatcctggccggccgggtctcaatggaatgaaaggagatcctggtctccctggtgttccaggattcccaggcatgaaaggacccagtggagtacctggatcagctggccctgagggggaaccgggacttattggtcctccaggtcctcctggattacctggtccttcaggacagagtatcataattaaaggagatgctggtcctccaggaatccctggccagcctgggctaaagggtctaccaggaccccaaggacctcaaggcttaccaggtccaactggccctccaggagatcctggacgcaatggactccctggctttgatggtgcaggagggcgcaaaggagacccaggtctgccaggacagccaggtacccgtggtttggatggtccccctggtccagatggattgcaaggtcccccaggtccccctggaacctcctctgttgcacatggatttcttattacacgccacagccagacaacggatgcaccacaatgcccacagggaacacttcaggtctatgaaggcttttctctcctgtatgtacaaggaaataaaagagcccacggtcaagacttggggacggctggcagctgccttcgtcgctttagtaccatgcctttcatgttctgcaacatcaataatgtttgcaactttgcttcaagaaatgactattcttactggctctctaccccagagcccatgccaatgagcatgcaacccctaaagggccagagcatccagccattcattagtcgatgtgcagtatgtgaagctccagctgtggtgatcgcagttcacagtcagacgatccagattccccattgtcctcagggatgggattctctgtggattggttattccttcatgatgcatacaagtgcaggggcagaaggctcaggtcaagccctagcctcccctggttcctgcttggaagagtttcgttcagctcccttcatcgaatgtcatgggaggggtacctgtaactactatgccaactcctacagcttttggctggcaactgtagatgtgtcagacatgttcagtaaacctcagtcagaaacgctgaaagcaggagacttgaggacacgaattagccgatgtcaagtgtgcatgaagaggacataa

SEQ ID NO: 27 - DNA, 186 bp, unidentified
  misc_feature 1..186: note = Exemplary NPHS1 enhancer
  source 1..186: mol_type = other DNA
ctgctgagctgggagaccaccttgatctgacttctcccatcttcccagcctaagccaggccctggggtcacggaggctggggaggcaccgaggaacgcgcctggcatgtgctgacaggggattttatgctccagctgggccagctgggaggagcctgctgggcagaggccagagctgggggctctg

SEQ ID NO: 28 - RNA, 13 nt, unidentified
  source 1..13: mol_type = other RNA
gccgccaccatgg

SEQ ID NO: 29 - DNA, 589 bp, unidentified
  misc_feature 1..589: note = Exemplary WPRE
  source 1..589: mol_type = other DNA
aatcaacctctggattacaaaatttgtgaaagattgactggtattcttaactatgttgctccttttacgctatgtggatacgctgctttaatgcctttgtatcatgctattgcttcccgtatggctttcattttctcctccttgtataaatcctggttgctgtctctttatgaggagttgtggcccgttgtcaggcaacgtggcgtggtgtgcactgtgtttgctgacgcaacccccactggttggggcattgccaccacctgtcagctcctttccgggactttcgctttccccctccctattgccacggcggaactcatcgccgcctgccttgcccgctgctggacaggggctcggctgttgggcactgacaattccgtggtgttgtcggggaaatcatcgtcctttccttggctgctcgcctgtgttgccacctggattctgcgcgggacgtccttctgctacgtcccttcggccctcaatccagcggaccttccttcccgcggcctgctgccggctctgcggcctcttccgcgtcttcgccttcgccctcagacgagtcggatctccctttgggccgcctccccgc

SEQ ID NO: 30 - DNA, 135 bp, unidentified
  misc_feature 1..135: note = Exemplary SV40pA signal sequence
  source 1..135: mol_type = other DNA
aacttgtttattgcagcttataatggttacaaataaagcaatagcatcacaaatttcacaaataaagcatttttttcactgcattctagttgtggtttgtccaaactcatcaatgtatcttatcatgtctggatc

SEQ ID NO: 31 - DNA, 225 bp, unidentified
  misc_feature 1..225: note = Exemplary bGH poly(A) signal sequence
  source 1..225: mol_type = other DNA
ctgtgccttctagttgccagccatctgttgtttgcccctcccccgtgccttccttgaccctggaaggtgccactcccactgtcctttcctaataaaatgaggaaattgcatcgcattgtctgagtaggtgtcattctattctggggggtggggtggggcaggacagcaagggggaggattgggaagacaatagcaggcatgctggggatgcggtgggctctatgg

SEQ ID NO: 32 - DNA, 17 bp, unidentified
  misc_feature 1..17: note = Exemplary soluble neuropilin-1 polyadenylation signal
  source 1..17: mol_type = other DNA
aaataaaatacgaaatg

SEQ ID NO: 33 - protein, 735 aa, unidentified
  REGION 1..735: note = Exemplary AAV3B VP1 capsid protein
MAADGYLPDWLEDNLSEGIREWWALKPGVPQPKANQQHQDNRRGLVLPGYKYLGPGNGLDKGEPVNEADAAALEHDKAYDQQLKAGDNPYLKYNHADAEFQERLQEDTSFGGNLGRAVFQAKKRILEPLGLVEEAAKTAPGKKRPVDQSPQEPDSSSGVGKSGKQPARKRLNFGQTGDSESVPDPQPLGEPPAAPTSLGSNTMASGGGAPMADNNEGADGVGNSSGNWHCDSQWLGDRVITTSTRTWALPTYNNHLYKQISSQSGASNDNHYFGYSTPWGYFDFNRFHCHFSPRDWQRLINNNWGFRPKKLSFKLFNIQVKEVTQNDGTTTIANNLTSTVQVFTDSEYQLPYVLGSAHQGCLPPFPADVFMVPQYGYLTLNNGSQAVGRSSFYCLEYFPSQMLRTGNNFQFSYTFEDVPFHSSYAHSQSLDRLMNPLIDQYLYYLNRTQGTTSGTTNQSRLLFSQAGPQSMSLQARNWLPGPCYRQQRLSKTANDNNNSNFPWTAASKYHLNGRDSLVNPGPAMASHKDDEEKFFPMHGNLIFGKEGTTASNAELDNVMITDEEEIRTTNPVATEQYGTVANNLQSSNTAPTTRTVNDQGALPGMVWQDRDVYLQGPIWAKIPHTDGHFHPSPLMGGFGLKHPPPQIMIKNTPVPANPPTTFSPAKFASFITQYSTGQVSVEIEWELQKENSKRWNPEIQYTSNYNKSVNVDFTVDTNGVYSEPRPIGTRYLTRN

SEQ ID NO: 34 - protein, 736 aa, unidentified
MAADGYLPDWLEDNLSEGIREWWALQPGAPKPKANQQHQDNARGLVLPGYKYLGPGNGLDKGEPVNAADAAALEHDKAYDQQLKAGDNPYLKYNHADAEFQERLKEDTSFGGNLGRAVFQAKKRLLEPLGLVEEAAKTAPGKKRPVDQSPQEPDSSSGVGKSGKQPARKRLNFGQTGDSESVPDPQPLGEPPAAPTSLGSNTMASGGGAPMADNNEGADGVGNSSGNWHCDSQWLGDRVITTSTRTWALPTYNNHLYKQISSQSGASNDNHYFGYSTPWGYFDFNRFHCHFSPRDWQRLINNNWGFRPKKLSFKLFNIQVKEVTQNDGTTTIANNLTSTVQVFTDSEYQLPYVLGSAHQGCLPPFPADVFMVPQYGYLTLNNGSQAVGRSSFYCLEYFPSQMLRTGNNFQFSYTFEDVPFHSSYAHSQSLDRLMNPLIDQYLYYLNRTQGTTSGTTNQSRLLFSQAGPQSMSLQARNWLPGPCYRQQRLSKTANDNNNSNFPWTAASKYHLNGRDSLVNPGPAMASHKDDEEKFFPMHGNLIFGKEGTTASNAELDNVMITDEEEIRTTNPVATEQYGTVANNLQSSNTAPTTRTVNDQGALPGMVWQDRDVYLQGPIWAKIPHTDGHFHPSPLMGGFGLKHPPPQIMIKNTPVPANPPTTFSPAKFASFITQYSTGQVSVEIEWELQKENSKRWNPEIQYTSNYNKSVNVDFTVDTNGVYSEPRPIGTRYLTRPL

SEQ ID NO: 35 - protein, 736 aa, unidentified
  REGION 1..736: note = Exemplary AAV9 VP1 capsid protein
MAADGYLPDWLEDNLSEGIREWWALKPGAPQPKANQQHQDNARGLVLPGYKYLGPGNGLDKGEPVNAADAAALEHDKAYDQQLKAGDNPYLKYNHADAEFQERLKEDTSFGGNLGRAVFQAKKRLLEPLGLVEEAAKTAPGKKRPVEQSPQEPDSSAGIGKSGAQPAKKRLNFGQTGDTESVPDPQPIGEPPAAPSGVGSLTMASGGGAPVADNNEGADGVGSSSGNWHCDSQWLGDRVITTSTRTWALPTYNNHLYKQISNSTSGGSSNDNAYFGYSTPWGYFDFNRFHCHFSPRDWQRLINNNWGFRPKRLNFKLFNIQVKEVTDNNGVKTIANNLTSTVQVFTDSDYQLPYVLGSAHEGCLPPFPADVFMIPQYGYLTLNDGSQAVGRSSFYCLEYFPSQMLRTGNNFQFSYEFENVPFHSSYAHSQSLDRLMNPLIDQYLYYLSKTINGSGQNQQTLKFSVAGPSNMAVQGRNYIPGPSYRQQRVSTTVTQNNNSEFAWPGASSWALNGRNSLMNPGPAMASHKEGEDRFFPLSGSLIFGKQGTGRDNVDADKVMITNEEEIKTTNPVATESYGQVATNHQSAQAQAQTGWVQNQGILPGMVWQDRDVYLQGPIWAKIPHTDGNFHPSPLMGGFGMKHPPPQILIKNTPVPADPPTAFNKDKLNSFITQYSTGQVSVEIEWELQKENSKRWNPEIQYTSNYYKSNNVEFAVNTEGVYSEPRPIGTRYLTRNL

SEQ ID NO: 36 - DNA, 1257 bp, unidentified
  misc_feature 1..1257: note = Exemplary VEGFC polynucleotide
  source 1..1257: mol_type = other DNA
atgcacttgctgggcttcttctctgtggcgtgttctctgctcgccgctgcgctgctcccgggtcctcgcgaggcgcccgccgccgccgccgccttcgagtccggactcgacctctcggacgcggagcccgacgcgggcgaggccacggcttatgcaagcaaagatctggaggagcagttacggtctgtgtccagtgtagatgaactcatgactgtactctacccagaatattggaaaatgtacaagtgtcagctaaggaaaggaggctggcaacataacagagaacaggccaacctcaactcaaggacagaagagactataaaatttgctgcagcacattataatacagagatcttgaaaagtattgataatgagtggagaaagactcaatgcatgccacgggaggtgtgtatagatgtggggaaggagtttggagtcgcgacaaacaccttctttaaacctccatgtgtgtccgtctacagatgtgggggttgctgcaatagtgaggggctgcagtgcatgaacaccagcacgagctacctcagcaagacgttatttgaaattacagtgcctctctctcaaggccccaaaccagtaacaatcagttttgccaatcacacttcctgccgatgcatgtctaaactggatgtttacagacaagttcattccattattagacgttccctgccagcaacactaccacagtgtcaggcagcgaacaagacctgccccaccaattacatgtggaataatcacatctgcagatgcctggctcaggaagattttatgttttcctcggatgctggagatgactcaacagatggattccatgacatctgtggaccaaacaaggagctggatgaagagacctgtcagtgtgtctgcagagcggggcttcggcctgccagctgtggaccccacaaagaactagacagaaactcatgccagtgtgtctgtaaaaacaaactcttccccagccaatgtggggccaaccgagaatttgatgaaaacacatgccagtgtgtatgtaaaagaacctgccccagaaatcaacccctaaatcctggaaaatgtgcctgtgaatgtacagaaagtccacagaaatgcttgttaaaaggaaagaagttccaccaccaaacatgcagctgttacagacggccatgtacgaaccgccagaaggcttgtgagccaggattttcatatagtgaagaagtgtgtcgttgtgtcccttcatattggaaaagaccacaaatgagc

SEQ ID NO: 37-41 - skipped (5 entries)

SEQ ID NO: 42 - DNA, 50 bp, unidentified
  misc_feature 1..50: note = Exemplary chicken beta-globin polyadenylation signal
  source 1..50: mol_type = other DNA
caataaaagatctttattttcattagatctgtgtgttggttttttgtgtg

SEQ ID NO: 43 - DNA, 30 bp, unidentified
  misc_feature 1..30: note = Exemplary transcription factor binding region
  source 1..30: mol_type = other DNA
gagcaagacagagagagatactcacaggga

SEQ ID NO: 44 - DNA, 1192 bp, unidentified
  misc_feature 1..1192: note = Exemplary variant nephrin promoter
  source 1..1192: mol_type = other DNA
cacctgaggtcaggagttcgagaccagcgtggccaacatgatgaaaccccgtctctagtaaaaatacaaaaattagccaggcatggtgctatatacctgtagcaccagctacttgggagacagaggtgggagaattacttgaacctgggaggttcaagccatgggaggtggaagttgcagtgagccgagatgccactgcactccagcctgagcaacagagcaagactatctcaagaaaagaaagaaagaaagaaagagacttgccaaggtcatgtatcagggcaaggaagagctgggggcccagctggctgctcccctgctgagctgggagaccaccttgatctgacttctcccatcttcccagcctaagccaggccctggggtcacggaggctggggaggcaccgaggaacgcgcctggcatgtgctgacagggaattttatgctccagctgggccagctgggaggagcctgctgggcagaggccagagctgggggctctggaaggtacctgggggaggttgcactgtgagaatgagctcaagctgggtcagagagcagggctgactctgccagtgcctgcatcagcctcatcgctctcctaggctcctggcctgctggactctgggctgcaggtccttcttgaaaggctgtgagtagtgagacaaggagcaggagtgaggggtggcaggagagaagatagagattgagagagagagagagagagagacagagagagaggaagagacagagacaaaaggagagagaacggcttagacaaggagagaaagatggaaagataaagagactgggcgcagtggctcacgcctgtaatcccaacacttggggaggccaaggtgggaggatggcttgaaggaaagagtctgagatcaacctggccaacatagtgagaccccgtctctaaaaaaaaaagaaaaaaaaaagaaaaaagaaaaaaaagtttttttaaagagacagagaaagagactcagagattgagactgagagcaagacagagagagacactcacagggaagaggggaagaggaaaacgagaaagggaggagagtaacggaaagagataaaaaagaaaagcaggtggcagagacacagagagagggacccagagaaagccagacagacgcaggtggctggcagcgggcgctgtgggggtcacagtagggggacctgtc

SEQ ID NO: 45 - DNA, 1192 bp, unidentified
  misc_feature 1..1192: note = Exemplary variant nephrin promoter
  source 1..1192: mol_type = other DNA
cacctgaggtcaggagttcgagaccagcgtggccaacatgatgaaaccccgtctctagtaaaaatacaaaaattagccaggcatggtgctatatacctgtagcaccagctacttgggagacagaggtgggagaattacttgaacctgggaggttcaagccatgggaggtggaagttgcagtgagccgagatgccactgcactccagcctgagcaacagagcaagactatctcaagaaaagaaagaaagaaagaaagagacttgccaaggtcatgtatcagggcaaggaagagctgggggcccagctggctgctcccctgctgagctgggagaccaccttgatctgacttctcccatcttcccagcctaagccaggccctggggtcacggaggctggggaggcaccgaggaacgcgcctggcatgtgctgacaggggattttatgctccagctgggccagctgggaggagcctgctgggcagaggccagagctgggggctctggaaggtacctgggggaggttgcactgtgagaatgagctcaagctgggtcagagagcagggctgactctgccagtgcctgcatcagcctcatcgctctcctaggctcctggcctgctggactctgggctgcaggtccttcttgaaaggctgtgagtagtgagacaaggagcaggagtgaggggtggcaggagagaagatagagattgagagagagagagagagagagacagagagagaggaagagacagagacaaaaggagagagaacggcttagacaaggagagaaagatggaaagataaagagactgggcgcagtggctcacgcctgtaatcccaacacttggggaggccaaggtgggaggatggcttgaaggaaagagtctgagatcaacctggccaacatagtgagaccccgtctctaaaaaaaaaagaaaaaaaaaagaaaaaagaaaaaaaagtttttttaaagagacagagaaagagactcagagattgagactgagagcaagacagagagagatactcacagggaagaggggaagaggaaaacgagaaagggaggagagtaacggaaagagataaaaaagaaaagcaggtggcagagacacagagagagggacccagagaaagccagacagacgcaggtggctggcagcgggcgctgtgggggtcacagtagggggacctgtc

SEQ ID NO: 46 - DNA, 819 bp, unidentified
  misc_feature 1..819: note = Exemplary minimal nephrin promoter variant
  source 1..819: mol_type = other DNA
ggccctggggtcacggaggctggggaggcaccgaggaacgcgcctggcatgtgctgacaggggattttatgctccagctgggccagctgggaggagcctgctgggcagaggccagagctgggggctctggaaggtacctgggggaggttgcactgtgagaatgagctcaagctgggtcagagagcagggctgactctgccagtgcctgcatcagcctcatcgctctcctaggctcctggcctgctggactctgggctgcaggtccttcttgaaaggctgtgagtagtgagacaaggagcaggagtgaggggtggcaggagagaagatagagattgagagagagagagagagagacagagagagaggaagagacagagacaaaaggagagagaacggcttagacaaggagagaaagatggaaagataaagagactgggcgcagtggctcacgcctgtaatcccaacacttggggaggccaaggtgggaggatggcttgaaggaaagagtctgagatcaacctggccaacatagtgagaccccgtctctaaaaaaaaaaaagaaaaaaaaaagaaaaaagaaaaaaaagtttttttaaagagacagagaaagagactcagagattgagactgagagcaagacagagagagatactcacagggaagaggggaagaggaaaacgagaaagggaggagagtaacggaaagagataaaaaagaaaagcaggtggcagagacacagagagagggacccagagaaagccagacagacgcaggtggctggcagcgggcgctgtgggggtcacagtagggggacctgtc

SEQ ID NO: 47 - DNA, 265 bp, unidentified
  misc_feature 1..265: note = Exemplary minimal nephrin promoter variant
  source 1..265: mol_type = other DNA
ggccctggggtcacggaggctggggaggcaccgaggaacgcgcctggcatgtgctgacaggggattttatgctccaggagcaagacagagagagatactcacagggaagaggggaagaggaaaacgagaaagggaggagagtaacggaaagagataaaaaagaaaagcaggtggcagagacacacagagagggacccagagaaagccagacagacgcaggtggctggcagcgggcgctgtgggggtcacagtagggggacctgtg

SEQ ID NO: 48 - skipped

SEQ ID NO: 49 - protein, 583 aa, unidentified
  REGION 1..583: note = Illustrative CFI polypeptide sequence
MKLLHVFLLFLCFHLRFCKVTYTSQEDLVEKKCLAKKYTHLSCDKVFCQPWQRCIEGTCVCKLPYQCPKNGTAVCATNRRSFPTYCQQKSLECLHPGTKFLNNGTCTAEGKFSVSLKHGNTDSEGIVEVKLVDQDKTMFICKSSWSMREANVACLDLGFQQGADTQRRFKLSDLSINSTECLHVHCRGLETSLAECTFTKRRTMGYQDFADVVCYTQKADSPMDDFFQCVNGKYISQMKACDGINDCGDQSDELCCKACQGKGFHCKSGVCIPSQYQCNGEVDCITGEDEVGCAGFASVTQEETEILTADMDAERRRIKSLLPKLSCGVKNRMHIRRKRIVGGKRAQLGDLPWQVAIKDASGITCGGIYIGGCWILTAAHCLRASKTHRYQIWTTVVDWIHPDLKRIVIEYVDRIIFHENYNAGTYQNDIALIEMKKDGNKKDCELPRSIPACVPWSPYLFQPNDTCIVSGWGREKDNERVFSLQWGEVKLISNCSKFYGNRFYEKEMECAGTYDGSIDACKGDSGGPLVCMDANNVTYVWGVVSWGENCGKPEFPGVYTKVANYFDWISYHVGRPFISQYNV

SEQ ID NO: 50 - DNA, 1752 bp, unidentified
  misc_feature 1..1752: note = Illustrative CFI polynucleotide sequence
  source 1..1752: mol_type = other DNA
atgaagcttcttcatgttttcctgttatttctgtgcttccacttaaggttttgcaaggtcacttatacatctcaagaggatctggtggagaaaaagtgcttagcaaaaaaatatactcacctctcctgcgataaagtcttctgccagccatggcagagatgcattgagggcacctgtgtttgtaaactaccgtatcagtgcccaaagaatggcactgcagtgtgtgcaactaacaggagaagcttcccaacatactgtcaacaaaagagtttggaatgtcttcatccagggacaaagtttttaaataacggaacatgcacagccgaaggaaagtttagtgtttccttgaagcatggaaatacagattcagagggaatagttgaagtaaaacttgtggaccaagataagacaatgttcatatgcaaaagcagctggagcatgagggaagccaacgtggcctgccttgaccttgggtttcaacaaggtgctgatactcaaagaaggtttaagttgtctgatctctctataaattccactgaatgtctacatgtgcattgccgaggattagagaccagtttggctgaatgtacttttactaagagaagaactatgggttaccaggatttcgctgatgtggtttgttatacacagaaagcagattctccaatggatgacttctttcagtgtgtgaatgggaaatacatttctcagatgaaagcctgtgatggtatcaatgattgtggagaccaaagtgatgaactgtgttgtaaagcatgccaaggcaaaggcttccattgcaaatcgggtgtttgcattccaagccagtatcaatgcaatggtgaggtggactgcattacaggggaagatgaagttggctgtgcaggctttgcatctgtgactcaagaagaaacagaaattttgactgctgacatggatgcagaaagaagacggataaaatcattattacctaaactatcttgtggagttaaaaacagaatgcacattcgaaggaaacgaattgtgggaggaaagcgagcacaactgggagacctcccatggcaggtggcaattaaggatgccagtggaatcacctgtgggggaatttatattggtggctgttggattctgactgctgcacattgtctcagagccagtaaaactcatcgttaccaaatatggacaacagtagtagactggatacaccccgaccttaaacgtatagtaattgaatacgtggatagaattattttccatgaaaactacaatgcaggcacttaccaaaatgacatcgctttgattgaaatgaaaaaagacggaaacaaaaaagattgtgagctgcctcgttccatccctgcctgtgtcccctggtctccttacctattccaacctaatgatacatgcatcgtttctggctggggacgagaaaaagataacgaaagagtcttttcacttcagtggggtgaagttaaactaataagcaactgctctaagttttacggaaatcgtttctatgaaaaagaaatggaatgtgcaggtacatatgatggttccatcgatgcctgtaaaggggactctggaggccccttagtctgtatggatgccaacaatgtgacttatgtctggggtgttgtgagttggggggaaaactgtggaaaaccagagttcccaggtgtttacaccaaagtggccaattattttgactggattagctaccatgtaggaaggccttttatttctcagtacaatgtataa

SEQ ID NO: 51 - protein, 1231 aa, unidentified
  REGION 1..1231: note = Illustrative CFH polypeptide sequence
MRLLAKIICLMLWAICVAEDCNELPPRRNTEILTGSWSDQTYPEGTQAIYKCRPGYRSLGNVIMVCRKGEWVALNPLRKCQKRPCGHPGDTPFGTFTLTGGNVFEYGVKAVYTCNEGYQLLGEINYRECDTDGWTNDIPICEVVKCLPVTAPENGKIVSSAMEPDREYHFGQAVRFVCNSGYKIEGDEEMHCSDDGFWSKEKPKCVEISCKSPDVINGSPISQKIIYKENERFQYKCNMGYEYSERGDAVCTESGWRPLPSCEEKSCDNPYIPNGDYSPLRIKHRTGDEITYQCRNGFYPATRGNTAKCTSTGWIPAPRCTLKPCDYPDIKHGGLYHENMRRPYFPVAVGKYYSYYCDEHFETPSGSYWDHIHCTQDGWSPAVPCLRKCYFPYLENGYNQNYGRKFVQGKSIDVACHPGYALPKAQTTVTCMENGWSPTPRCIRVKTCSKSSIDIENGFISESQYTYALKEKAKYQCKLGYVTADGETSGSITCGKDGWSAQPTCIKSCDIPVFMNARTKNDFTWFKLNDTLDYECHDGYESNTGSTTGSIVCGYNGWSDLPICYERECELPKIDVHLVPDRKKDQYKVGEVLKFSCKPGFTIVGPNSVQCYHFGLSPDLPICKEQVQSCGPPPELLNGNVKEKTKEEYGHSEVVEYYCNPRFLMKGPNKIQCVDGEWTTLPVCIVEESTCGDIPELEHGWAQLSSPPYYYGDSVEFNCSESFTMIGHRSITCIHGVWTQLPQCVAIDKLKKCKSSNLIILEEHLKNKKEFDHNSNIRYRCRGKEGWIHTVCINGRWDPEVNCSMAQIQLCPPPPQIPNSHNMTTTLNYRDGEKVSVLCQENYLIQEGEEITCKDGRWQSIPLCVEKIPCSQPPQIEHGTINSSRSSQESYAHGTKLSYTCEGGFRISEENETTCYMGKWSSPPQCEGLPCKSPPEISHGVVAHMSDSYQYGEEVTYKCFEGFGIDGPAIAKCLGEKWSHPPSCIKTDCLSLPSFENAIPMGEKKDVYKAGEQVTYTCATYYKMDGASNVTCINSRWTGRPTCRDTSCVNPPTVQNAYIVSRQMSKYPSGERVRYQCRSPYEMFGDEEVMCLNGNWTEPPQCKDSTGKCGPPPPIDNGDITSFPLSVYAPASSVEYQCQNLYQLEGNKRITCRNGQWSEPPKCLHPCVISREIMENYNIALRWTAKQKLYSRTGESVEFVCKRGYRLSSRSHTLRTTCWDGKLEYPTCAKR

SEQ ID NO: 52 - DNA, 3696 bp, unidentified
  misc_feature 1..3696: note = Illustrative CFH polynucleotide sequence
  source 1..3696: mol_type = other DNA
atgagacttctagcaaagattatttgccttatgttatgggctatttgtgtagcagaagattgcaatgaacttcctccaagaagaaatacagaaattctgacaggttcctggtctgaccaaacatatccagaaggcacccaggctatctataaatgccgccctggatatagatctcttggaaatgtaataatggtatgcaggaagggagaatgggttgctcttaatccattaaggaaatgtcagaaaaggccctgtggacatcctggagatactccttttggtacttttacccttacaggaggaaatgtgtttgaatatggtgtaaaagctgtgtatacatgtaatgaggggtatcaattgctaggtgagattaattaccgtgaatgtgacacagatggatggaccaatgatattcctatatgtgaagttgtgaagtgtttaccagtgacagcaccagagaatggaaaaattgtcagtagtgcaatggaaccagatcgggaataccattttggacaagcagtacggtttgtatgtaactcaggctacaagattgaaggagatgaagaaatgcattgttcagacgatggtttttggagtaaagagaaaccaaagtgtgtggaaatttcatgcaaatccccagatgttataaatggatctcctatatctcagaagattatttataaggagaatgaacgatttcaatataaatgtaacatgggttatgaatacagtgaaagaggagatgctgtatgcactgaatctggatggcgtccgttgccttcatgtgaagaaaaatcatgtgataatccttatattccaaatggtgactactcacctttaaggattaaacacagaactggagatgaaatcacgtaccagtgtagaaatggtttttatcctgcaacccggggaaatacagcaaaatgcacaagtactggctggatacctgctccgagatgtaccttgaaaccttgtgattatccagacattaaacatggaggtctatatcatgagaatatgcgtagaccatactttccagtagctgtaggaaaatattactcctattactgtgatgaacattttgagactccgtcaggaagttactgggatcacattcattgcacacaagatggatggtcgccagcagtaccatgcctcagaaaatgttattttccttatttggaaaatggatataatcaaaatcatggaagaaagtttgtacagggtaaatctatagacgttgcctgccatcctggctacgctcttccaaaagcgcagaccacagttacatgtatggagaatggctggtctcctactcccagatgcatccgtgtcaaaacatgttccaaatcaagtatagatattgagaatgggtttatttctgaatctcagtatacatatgccttaaaagaaaaagcgaaatatcaatgcaaactaggatatgtaacagcagatggtgaaacatcaggatcaattacatgtgggaaagatggatggtcagctcaacccacgtgcattaaatcttgtgatatcccagtatttatgaatgccagaactaaaaatgacttcacatggtttaagctgaatgacacattggactatgaatgccatgatggttatgaaagcaatactggaagcaccactggttccatagtgtgtggttacaatggttggtctgatttacccatatgttatgaaagagaatgcgaacttcctaaaatagatgtacacttagttcctgatcgcaagaaagaccagtataaagttggagaggtgttgaaattctcctgcaaaccaggatttacaatagttggacctaattccgttcagtgctaccactttggattgtctcctgacctcccaatatgtaaagagcaagtacaatcatgtggtccacctcctgaactcctcaatgggaatgttaaggaaaaaacgaaagaagaatatggacacagtgaagtggtggaatattattgcaatcctagatttctaatgaagggacctaataaaattcaatgtgttgatggagagtggacaactttaccagtgtgtattgtggaggagagtacctgtggagatatacctgaacttgaacatggctgggcccagctttcttcccctccttattactatggagattcagtggaattcaattgctcagaatcatttacaatgattggacacagatcaattacgtgtattcatggagtatggacccaacttccccagtgtgtggcaatagataaacttaagaagtgcaaatcatcaaatttaattatacttgaggaacatttaaaaaacaagaaggaattcgatcataattctaacataaggtacagatgtagaggaaaagaaggatggatacacacagtctgcataaatggaagatgggatccagaagtgaactgctcaatggcacaaatacaattatgcccacctccacctcagattcccaattctcacaatatgacaaccacactgaattatcgggatggagaaaaagtatctgttctttgccaagaaaattatctaattcaggaaggagaagaaattacatgcaaagatggaagatggcagtcaataccactctgtgttgaaaaaattccatgttcacaaccacctcagatagaacacggaaccattaattcatccaggtcttcacaagaaagttatgcacatgggactaaattgagttatacttgtgagggtggtttcaggatatctgaagaaaatgaaacaacatgctacatgggaaaatggagttctccacctcagtgtgaaggccttccttgtaaatctccacctgagatttctcatggtgttgtagctcacatgtcagacagttatcagtatggagaagaagttacgtacaaatgttttgaaggttttggaattgatgggcctgcaattgcaaaatgcttaggagaaaaatggtctcaccctccatcatgcataaaaacagattgtctcagtttacctagctttgaaaatgccatacccatgggagagaagaaggatgtgtataaggcgggtgagcaagtgacttacacttgtgcaacatattacaaaatggatggagccagtaatgtaacatgcattaatagcagatggacaggaaggccaacatgcagagacacctcctgtgtgaatccgcccacagtacaaaatgcttatatagtgtcgagacagatgagtaaatatccatctggtgagagagtacgttatcaatgtaggagcccttatgaaatgtttggggatgaagaagtgatgtgtttaaatggaaactggacggaaccacctcaatgcaaagattctacaggaaaatgtgggccccctccacctattgacaatggggacattacttcattcccgttgtcagtatatgctccagcttcatcagttgagtaccaatgccagaacttgtatcaacttgagggtaacaagcgaataacatgtagaaatggacaatggtcagaaccaccaaaatgcttacatccgtgtgtaatatcccgagaaattatggaaaattataacatagcattaaggtggacagccaaacagaagctttattcgagaacaggtgaatcagttgaatttgtgtgtaaacggggatatcgtctttcatcacgttctcacacattgcgaacaacatgttgggatgggaaactggagtatccaacttgtgcaaaaagatag

SEQ ID NO: 53 - protein, 449 aa, unidentified
  REGION 1..449: note = Illustrative FHL-1 polypeptide sequence
MRLLAKIICLMLWAICVAEDCNELPPRRNTEILTGSWSDQTYPEGTQAIYKCRPGYRSLGNVIMVCRKGEWVALNPLRKCQKRPCGHPGDTPFGTFTLTGGNVFEYGVKAVYTCNEGYQLLGEINYRECDTDGWTNDIPICEVVKCLPVTAPENGKIVSSAMEPDREYHFGQAVRFVCNSGYKIEGDEEMHCSDDGFWSKEKPKCVEISCKSPDVINGSPISQKIIYKENERFQYKCNMGYEYSERGDAVCTESGWRPLPSCEEKSCDNPYIPNGDYSPLRIKHRTGDEITYQCRNGFYPATRGNTAKCTSTGWIPAPRCTLKPCDYPDIKHGGLYHENMRRPYFPVAVGKYYSYYCDEHFETPSGSYWDHIHCTQDGWSPAVPCLRKCYFPYLENGYNQNHGRKFVQGKSIDVACHPGYALPKAQTTVTCMENGWSPTPRCIRVSFTL

SEQ ID NO: 54 - DNA, 1350 bp, unidentified
  misc_feature 1..1350: note = Illustrative FHL-1 polynucleotide sequence
  source 1..1350: mol_type = other DNA
atgagacttctagcaaagattatttgccttatgttatgggctatttgtgtagcagaagattgcaatgaacttcctccaagaagaaatacagaaattctgacaggttcctggtctgaccaaacatatccagaaggcacccaggctatctataaatgccgccctggatatagatctcttggaaatgtaataatggtatgcaggaagggagaatgggttgctcttaatccattaaggaaatgtcagaaaaggccctgtggacatcctggagatactccttttggtacttttacccttacaggaggaaatgtgtttgaatatggtgtaaaagctgtgtatacatgtaatgaggggtatcaattgctaggtgagattaattaccgtgaatgtgacacagatggatggaccaatgatattcctatatgtgaagttgtgaagtgtttaccagtgacagcaccagagaatggaaaaattgtcagtagtgcaatggaaccagatcgggaataccattttggacaagcagtacggtttgtatgtaactcaggctacaagattgaaggagatgaagaaatgcattgttcagacgatggtttttggagtaaagagaaaccaaagtgtgtggaaatttcatgcaaatccccagatgttataaatggatctcctatatctcagaagattatttataaggagaatgaacgatttcaatataaatgtaacatgggttatgaatacagtgaaagaggagatgctgtatgcactgaatctggatggcgtccgttgccttcatgtgaagaaaaatcatgtgataatccttatattccaaatggtgactactcacctttaaggattaaacacagaactggagatgaaatcacgtaccagtgtagaaatggtttttatcctgcaacccggggaaatacagcaaaatgcacaagtactggctggatacctgctccgagatgtaccttgaaaccttgtgattatccagacattaaacatggaggtctatatcatgagaatatgcgtagaccatactttccagtagctgtaggaaaatattactcctattactgtgatgaacattttgagactccgtcaggaagttactgggatcacattcattgcacacaagatggatggtcgccagcagtaccatgcctcagaaaatgttattttccttatttggaaaatggatataatcaaaatcatggaagaaagtttgtacagggtaaatctatagacgttgcctgccatcctggctacgctcttccaaaagcgcagaccacagttacatgtatggagaatggctggtctcctactcccagatgcatccgtgtcagctttaccctctga

SEQ ID NO: 55 - protein, 383 aa, unidentified
  REGION 1..383: note = Exemplary NPHS2 amino acid sequence
MERRARSSSRESRGRGGRTPHKENKRAKAERSGGGRGRQEAGPEPSGSGRAGTPGEPRAPAATVVDVDEVRGSGEEGTEVVALLESERPEEGTKSSGLGACEWLLVLISLLFIIMTFPFSIWFCVKVVQEYERVIIFRLGHLLPGRAKGPGLFFFLPCLDTYHKVDLRLQTLEIPFHEIVTKDMFIMEIDAICYYRMENASLLLSSLAHVSKAVQFLVQTTMKRLLAHRSLTEILLERKSIAQDAKVALDSVTCIWGIKVERIEIKDVRLPAGLQHSLAVEAEAQRQAKVRMIAAEAEKAASESLRMAAEILSGTPAAVQLRYLHTLQSLSTEKPSTVVLPLPFDLLNCLSSPSNRTQGSLPFPSPSKPVEPLNPKKKDSPML

SEQ ID NO: 56 - DNA, 1149 bp, unidentified
  misc_feature 1..1149: note = Exemplary NPHS2 transgene sequence
  source 1..1149: mol_type = other DNA
atggagaggagggcgcggagctcctccagggagtcccgcgggcgaggcggcaggactccgcacaaggagaacaagagggcaaaggccgagaggagcggcgggggccgcgggcgccaggaggctgggcccgagccgtcgggctccggacgggcggggaccccgggggagccccgagcgcccgccgccacggtggtggacgtggatgaggtccgaggctccggcgaggagggcaccgaggtggtggcgctgttggagagcgagcggcccgaggaaggtaccaaatcctccggcttaggggcctgtgagtggcttcttgtcctcatttccctgctcttcatcatcatgaccttccctttttccatctggttctgcgtaaaggttgtacaagagtatgaaagagtaattatattccgactgggacatctgcttcctggaagagccaaaggccctggtcttttcttttttttgccctgcctggatacctaccacaaggttgaccttcgtctccaaactctggagataccttttcatgagatcgtgaccaaagacatgtttataatggagatagatgccatttgctactaccgaatggaaaatgcctctcttctcctaagcagtcttgctcatgtatctaaagctgtgcaattccttgtgcaaaccactatgaagcgtctcctagcacatcgatccctcactgaaattcttctagagaggaagagcatcgcccaagatgcaaaggttgccttggattcagtgacctgtatttggggaatcaaagtggagagaatagaaattaaagatgtgaggttgccagctgggcttcagcactcactggctgtggaggctgaagcgcaaagacaagccaaagtgcggatgattgctgcagaagcggaaaaggctgcttctgagtccctgaggatggcagctgagattctgtcaggcacccctgctgctgttcagcttcgatacctccacacccttcagtctctgtccacagagaagccttccactgtggttttacctttgccatttgacctactgaattgcctgtcttctcccagcaacagaactcagggaagcctccccttcccaagtccttccaaacctgttgagccactaaatcctaaaaagaaagactctcccatgtta

SEQ ID NO: 57 - DNA, 1152 bp, unidentified
  misc_feature 1..1152: note = Exemplary NPHS2 transgene sequence
  source 1..1152: mol_type = other DNA
atggagaggagggcgcggagctcctccagggagtcccgcgggcgaggcggcaggactccgcacaaggagaacaagagggcaaaggccgagaggagcggcggaggccgcgggcgccaggaggctgggcccgagccgtcgggctccggacgggcggggaccccgggggagccccgagcgcccgccgccacggtggtggacgtggatgaggtccgaggctccggcgaggagggcaccgaggtggtggcgctgttggagagcgagcggcccgaggaaggtaccaaatcctccggcttaggggcctgtgagtggcttcttgtcctcatttccctgctcttcatcatcatgaccttccctttttccatctggttctgcgtaaaggttgtacaagagtatgaaagagtaattatattccgactgggacatctgcttcctggaagagccaaaggccctggtcttttcttttttttgccctgcctggatacctaccacaaggttgaccttcgtctccaaactctggagataccttttcatgagatcgtgaccaaagacatgtttataatggagatagatgccatttgctactaccgaatggaaaatgcctctcttctcctaagcagtcttgctcatgtatctaaagctgtgcaattccttgtgcaaaccactatgaagcgtctcctagcacatcgatccctcactgaaattcttctagagaggaagagcatcgcccaagatgcaaaggttgccttggattcagtgacctgtatttggggaatcaaagtggagagaatagaaattaaagatgtgaggttgccagctgggcttcagcactcactggctgtggaggctgaagcgcaaagacaagccaaagtgcggatgattgctgcagaagcggaaaaggctgcttctgagtccctgaggatggcagctgagattctgtcaggcacccctgctgccgttcagcttcgatacctccacacccttcagtctctgtccacagagaagccttccactgtggttttacctttgccatttgacctactgaattgcctgtcttctcccagcaacagaactcagggaagcctccccttcccaagtccttccaaacctgttgagccactaaatcctaaaaagaaagactctcccatgttatag

SEQ ID NO: 58 - DNA, 818 bp, unidentified
  misc_feature 1..818: note = Exemplary minimal nephrin promoter
  source 1..818: mol_type = other DNA
ggccctggggtcacggaggctggggaggcaccgaggaacgcgcctggcatgtgctgacagggaattttatgctccagctgggccagctgggaggagcctgctgggcagaggccagagctgggggctctggaaggtacctgggggaggttgcactgtgagaatgagctcaagctgggtcagagagcagggctgactctgccagtgcctgcatcagcctcatcgctctcctaggctcctggcctgctggactctgggctgcaggtccttcttgaaaggctgtgagtagtgagacaaggagcaggagtgaggggtggcaggagagaagatagagattgagagagagagagagagagacagagagagaggaagagacagagacaaaaggagagagaacggcttagacaaggagagaaagatggaaagataaagagactgggcgcagtggctcacgcctgtaatcccaacacttggggaggccaaggtgggaggatggcttgaaggaaagagtctgagatcaacctggccaacatagtgagaccccgtctctaaaaaaaaaaaagaaaaaaaaaagaaaaaagaaaaaaaagtttttttaaagagacagagaaagagactcagagattgagactgagagcaagacagagagagacactcacagggaagaggggaagaggaaaacgagaaagggaggagagtaacggaaagagataaaaaagaaaagcaggtggcagagacacagagagagggacccagagaaagccagacagacgcaggtggctggcagcgggcgctgtgggggtcacagtagggggacctgt

SEQ ID NO: 59 - DNA, 818 bp, unidentified
  misc_feature 1..818: note = Exemplary minimal nephrin promoter variant
  source 1..818: mol_type = other DNA
ggccctggggtcacggaggctggggaggcaccgaggaacgcgcctggcatgtgctgacaggggattttatgctccagctgggccagctgggaggagcctgctgggcagaggccagagctgggggctctggaaggtacctgggggaggttgcactgtgagaatgagctcaagctgggtcagagagcagggctgactctgccagtgcctgcatcagcctcatcgctctcctaggctcctggcctgctggactctgggctgcaggtccttcttgaaaggctgtgagtagtgagacaaggagcaggagtgaggggtggcaggagagaagatagagattgagagagagagagagagagagacagagagagaggaagagacagagacaaaaggagagagaacggcttagacaaggagagaaagatggaaagataaagagactgggcgcagtggctcacgcctgtaatcccaacacttggggaggccaaggtgggaggatggcttgaaggaaagagtctgagatcaacctggccaacatagtgagaccccgtctctaaaaaaaaaagaaaaaaaaaagaaaaaagaaaaaaaagtttttttaaagagacagagaaagagactcagagattgagactgagagcaagacagagagagatactcacagggaagaggggaagaggaaaacgagaaagggaggagagtaacggaaagagataaaaaagaaaagcaggtggcagagacacacagagagggacccagagaaagccagacagacgcaggtggctggcagcgggcgctgtgggggtcacagtagggggacctgt

SEQ ID NO: 60 - DNA, 818 bp, unidentified
  misc_feature 1..818: note = Exemplary minimal nephrin promoter variant
  source 1..818: mol_type = other DNA
ggccctggggtcacggaggctggggaggcaccgaggaacgcgcctggcatgtgctgacaggggattttatgctccagctgggccagctgggaggagcctgctgggcagaggccagagctgggggctctggaaggtacctgggggaggttgcactgtgagaatgagctcaagctgggtcagagagcagggctgactctgccagtgcctgcatcagcctcatcgctctcctaggctcctggcctgctggactctgggctgcaggtccttcttgaaaggctgtgagtagtgagacaaggagcaggagtgaggggtggcaggagagaagatagagattgagagagagagagagagagacagagagagaggaagagacagagacaaaaggagagagaacggcttagacaaggagagaaagatggaaagataaagagactgggcgcagtggctcacgcctgtaatcccaacacttggggaggccaaggtgggaggatggcttgaaggaaagagtctgagatcaacctggccaacatagtgagaccccgtctctaaaaaaaaaaaagaaaaaaaaaagaaaaaagaaaaaaaagtttttttaaagagacagagaaagagactcagagattgagactgagagcaagacagagagagatactcacagggaagaggggaagaggaaaacgagaaagggaggagagtaacggaaagagataaaaaagaaaagcaggtggcagagacacagagagagggacccagagaaagccagacagacgcaggtggctggcagcgggcgctgtgggggtcacagtagggggacctgt

SEQ ID NO: 61 - skipped

SEQ ID NO: 62 - DNA, 17 bp, unidentified
  misc_feature 1..17: note = sequence
  source 1..17: mol_type = other DNA
cggaggctggggaggca

SEQ ID NO: 63 - skipped